European Patent Specification EP 4 456 712 B1, published October 29, 2025. Title: PRODUCTS AND METHODS FOR IMPROVING PLANT GROWTH FEATURES. Applicant: Aphea.Bio NV. The sequence listing filed with the application follows.

SEQUENCE LISTING (3 sequences)

SEQ ID NO: 1 - DNA, 502 bp, Penicillium bialowiezense
  source 1..502: mol_type = genomic DNA
tatttaccttgttgcttcggcgagcctgccttttggctgccgggggacgtcagtccccgggtccgtgctcgccggagacaccttagaactctgtctgaagattgtagtctgagattaaatataaattatttaaaactttcaacaacggatctcttggttccggcatcgatgaagaacgcagcgaaatgcgatacgtaatgtgaattgcagaattcagtgaatcatcgagtctttgaacgcacattgcgccctctggtattccggagggcatgcctgtccgagcgtcattgctgccctcaagcacggcttgtgtgttgggccccgtcctccttccgggggacgggtccgaaaggcagcggcggcaccgcgtccggtcctcaagcgtatggggctttgtcactcgctttgtaggcctggccggcgcttgccgatcaaccaaactttttatcaggttgacctcggatcaggtagggatacccgctgaacttaagcatatcaaagg

SEQ ID NO: 2 - DNA, 19 bp, synthetic construct
  misc_feature 1..19: note = ITS forward primer
  source 1..19: mol_type = other DNA
tccgtaggtgaacctgcgg

SEQ ID NO: 3 - DNA, 20 bp, synthetic construct
  misc_feature 1..20: note = ITS reverse primer
  source 1..20: mol_type = other DNA
tcctccgcttattgatatgc